European Patent Application EP 4 186 925 A1, published May 31, 2023. Title: D8 BINDING POLYPEPTIDE AND USE THEREOF. Applicant: SUZHOU SMARTNUCLIDE BIOPHARMACEUTICAL CO., LTD. The sequence listing filed with the application follows.

SEQUENCE LISTING (91 sequences)

SEQ ID NO: 1 - protein, 409 aa, Artificial sequence
  Artificial sequence
MALPVTALLLPLALLLHAARPSQFRVSPLDRTWNLGETVELKCQVLLSNPTSGCSWLFQPRGAAASPTFLLYLSQNKPKAAEGLDTQRFSGKRLGDTFVLTLSDFRRENEGYYFCSALSNSIMYFSHFVPVFLPAKPTTTPAPRPPTPAPTIASQPLSLRPEACRPAAGGAGIEGRMDPKSSDKTHTCPPCPAPELLGGPSVFLFPPKPKDTLMISRTPEVTCVVVDVSHEDPEVKFNWYVDGVEVHNAKTKPREEQYNSTYRVVSVLTVLHQDWLNGKEYKCKVSNKALPAPIEKTISKAKGQPREPQVYTLPPSRDELTKNQVSLTCLVKGFYPSDIAVEWESNGQPENNYKTTPPVLDSDGSFFLYSKLTVDKSRWQQGNVFSCSVMHEALHNHYTQKSLSLSPGK

SEQ ID NO: 2 - protein, 10 aa, Artificial sequence
  Artificial sequence
GFTLDYYAIG

SEQ ID NO: 3 - protein, 17 aa, Artificial sequence
  Artificial sequence
CIRIYDGNTYSAESVKG

SEQ ID NO: 4 - protein, 16 aa, Artificial sequence
  Artificial sequence
GSYYSCSVYPDYDMDY

SEQ ID NO: 5 - protein, 125 aa, Artificial sequence
  Artificial sequence
QVQLVESGGGLVQPGGSLRLSCAASGFTLDYYAIGWFRQAPGKEREGISCIRIYDGNTYSAESVKGRFTISSDNAKNQVYLQINTLKPEDTAVYYCAAGSYYSCSVYPDYDMDYWGKGTLVTVSS

SEQ ID NO: 6 - protein, 10 aa, Artificial sequence
  Artificial sequence
GSIFSINTMG

SEQ ID NO: 7 - protein, 16 aa, Artificial sequence
  Artificial sequence
TMHSTGSTNYADSVKG

SEQ ID NO: 8 - protein, 10 aa, Artificial sequence
  Artificial sequence
DDTGWGTVDS

SEQ ID NO: 9 - protein, 117 aa, Artificial sequence
  Artificial sequence
QVQLVESGGGLVQPGGSLRLSCAASGSIFSINTMGWYRQAPGKQRELVATMHSTGSTNYADSVKGRFTISRDNAKKTVYLQMNSLEPDDTAVYYCHVDDTGWGTVDSWGQGTQVTVS

SEQ ID NO: 10 - protein, 10 aa, Artificial sequence
  Artificial sequence
GPIFSINTMG

SEQ ID NO: 11 - protein, 16 aa, Artificial sequence
  Artificial sequence
TMHSTGSTNYADSVKG

SEQ ID NO: 12 - protein, 10 aa, Artificial sequence
  Artificial sequence
DDTGWGTVDS

SEQ ID NO: 13 - protein, 118 aa, Artificial sequence
  Artificial sequence
QVQLVESGGGLVQPGGSLRLSCAASGPIFSINTMGWYRQAPGKQRELVATMHSTGSTNYADSVKGRFTISRDNAKKTVYLQMNSLKPDDTAVYYCHVDDTGWGTVDSWGQGIQVTVSS

SEQ ID NO: 14 - protein, 10 aa, Artificial sequence
  Artificial sequence
GSIFAINTMG

SEQ ID NO: 15 - protein, 16 aa, Artificial sequence
  Artificial sequence
TMHSGGSTNYADSVKG

SEQ ID NO: 16 - protein, 10 aa, Artificial sequence
  Artificial sequence
DDSGWGTVDS

SEQ ID NO: 17 - protein, 118 aa, Artificial sequence
  Artificial sequence
QLQLVESGGGLVQPGGSLRLSCVVSGSIFAINTMGWYRQAPGKQRELVATMHSGGSTNYADSVKGRFTISRDAAPKTVYLQMNSLKPADTAVYYCHADDSGWGTVDSWGQGIQVTVSS

SEQ ID NO: 18 - protein, 10 aa, Artificial sequence
  Artificial sequence
GFTSDDYVIG

SEQ ID NO: 19 - protein, 17 aa, Artificial sequence
  Artificial sequence
CISSSDGTTNYADSVKG

SEQ ID NO: 20 - protein, 21 aa, Artificial sequence
  Artificial sequence
DPMRVCPYSGTYYGILGFGTS

SEQ ID NO: 21 - protein, 129 aa, Artificial sequence
  Artificial sequence
QVQLVESGGGLVQAGGSLRLSCVASGFTSDDYVIGWFRQAPGKEREGVSCISSSDGTTNYADSVKGRFTISSDNAKNTVYLQMNSLKPEDTAVYYCAADPMRVCPYSGTYYGILGFGTSGQGTQVTVSS

SEQ ID NO: 22 - protein, 10 aa, Artificial sequence
  Artificial sequence
GSIFAINTMG

SEQ ID NO: 23 - protein, 16 aa, Artificial sequence
  Artificial sequence
DMHSTGSTNYADSVKG

SEQ ID NO: 24 - protein, 10 aa, Artificial sequence
  Artificial sequence
DDRGWGTVDS

SEQ ID NO: 25 - protein, 118 aa, Artificial sequence
  Artificial sequence
QVQLVESGGGLVQPGGSLRLSCVASGSIFAINTMGWYRQAPGKQRELVADMHSTGSTNYADSVKGRFTISRDNAKKKVYLQMNSLKPDDTAVYYCHVDDRGWGTVDSWGQGTQVTVSS

SEQ ID NO: 26 - protein, 10 aa, Artificial sequence
  Artificial sequence
GLTFEDYAIG

SEQ ID NO: 27 - protein, 17 aa, Artificial sequence
  Artificial sequence
CIRIYDGNTYSAESVKG

SEQ ID NO: 28 - protein, 16 aa, Artificial sequence
  Artificial sequence
GSYYSCSVYPDYDMDY

SEQ ID NO: 29 - protein, 125 aa, Artificial sequence
  Artificial sequence
QLQLVESGGGLVQAGGSLRLSCAASGLTFEDYAIGWFRQAPGKEREGISCIRIYDGNTYSAESVKGRFTISSDNAKNQVYLQINTLKPEDTAVYYCAAGSYYSCSVYPDYDMDYWGKGTLVTVSS

SEQ ID NO: 30 - protein, 10 aa, Artificial sequence
  Artificial sequence
GLTFEDYAIG

SEQ ID NO: 31 - protein, 17 aa, Artificial sequence
  Artificial sequence
CIRIYDGNTYSAESVKG

SEQ ID NO: 32 - protein, 16 aa, Artificial sequence
  Artificial sequence
GSYYSCSVYPDYDMDY

SEQ ID NO: 33 - protein, 125 aa, Artificial sequence
  Artificial sequence
QVQLVESGGGLVQAGGSLRLSCAASGLTFEDYAIGWFRQAPGKEREGISCIRIYDGNTYSAESVKGRFTISSDNAKNQVYLQINTLKPEDTAVYYCAAGSYYSCSVYPDYDMDYWGKGTLVTVSS

SEQ ID NO: 34 - protein, 10 aa, Artificial sequence
  Artificial sequence
GPIFSINTMG

SEQ ID NO: 35 - protein, 16 aa, Artificial sequence
  Artificial sequence
TMHSTGSTNYADSVKG

SEQ ID NO: 36 - protein, 10 aa, Artificial sequence
  Artificial sequence
DDTGWGTVDS

SEQ ID NO: 37 - protein, 118 aa, Artificial sequence
  Artificial sequence
QVQLVESGGGLVQPGGSLRLSCAASGPIFSINTMGWYRQVPGKQRELVATMHSTGSTNYADSVKGRFTISRDNAKKTVYLQMNSLKPDDTAVYYCHVDDTGWGTVDSWGQGTQVTVSS

SEQ ID NO: 38 - protein, 10 aa, Artificial sequence
  Artificial sequence
GVTFDDLAIG

SEQ ID NO: 39 - protein, 17 aa, Artificial sequence
  Artificial sequence
TIGTSDGTAYYADSVKG

SEQ ID NO: 40 - protein, 16 aa, Artificial sequence
  Artificial sequence
DLDYGLGSLLPMGYDY

SEQ ID NO: 41 - protein, 125 aa, Artificial sequence
  Artificial sequence
QVQLVESGGGLVQAGGSLRLSCAASGVTFDDLAIGWFRQVPGKGREGVSTIGTSDGTAYYADSVKGRFTISSDNAKNTVYLQMNSLKPEDTAVYYCAVDLDYGLGSLLPMGYDYWGQGTQVTVSS

SEQ ID NO: 42 - protein, 10 aa, Artificial sequence
  Artificial sequence
GGTFSSTAMG

SEQ ID NO: 43 - protein, 17 aa, Artificial sequence
  Artificial sequence
AISWSGGYTYYADSVRG

SEQ ID NO: 44 - protein, 20 aa, Artificial sequence
  Artificial sequence
DISGLDTVAAGIFTEPNIDY

SEQ ID NO: 45 - protein, 129 aa, Artificial sequence
  Artificial sequence
QVQLVESGGGLVQAGGSLRVSCAASGGTFSSTAMGWFRQAPGKEREFVAAISWSGGYTYYADSVRGRFTISRDNALNTVSLQMNSLKPEDTAVYYCAADISGLDTVAAGIFTEPNIDYWGKGTLVTVSS

SEQ ID NO: 46 - protein, 10 aa, Artificial sequence
  Artificial sequence
GTIFSINTMG

SEQ ID NO: 47 - protein, 16 aa, Artificial sequence
  Artificial sequence
TITSSGSTKYADSVKG

SEQ ID NO: 48 - protein, 10 aa, Artificial sequence
  Artificial sequence
NDVGWGTVNA

SEQ ID NO: 49 - protein, 118 aa, Artificial sequence
  Artificial sequence
QVQLVESGGGLVQPGGSLRLSCAVSGTIFSINTMGWYRQVPGKQRELVATITSSGSTKYADSVKGRFTVSRDNAKRTVFLQMDSLKPEDTAVYYCHANDVGWGTVNAWGQGTLVTVSS

SEQ ID NO: 50 - protein, 10 aa, Artificial sequence
  Artificial sequence
GSIFSINGMG

SEQ ID NO: 51 - protein, 16 aa, Artificial sequence
  Artificial sequence
VITSGGKIDYLDSVKG

SEQ ID NO: 52 - protein, 11 aa, Artificial sequence
  Artificial sequence
YGDVRRGEVRW

SEQ ID NO: 53 - protein, 118 aa, Artificial sequence
  Artificial sequence
QLQLVESGGGLVQPGGSLRLSCAASGSIFSINGMGWYRQAPGKQREAVAVITSGGKIDYLDSVKGRFTISRDSAKNTVALQMNSLKPEDTAVYYCNAYGDVRRGEVRWGQGTQVTVSS

SEQ ID NO: 54 - protein, 10 aa, Artificial sequence
  Artificial sequence
GSIFAINTMG

SEQ ID NO: 55 - protein, 16 aa, Artificial sequence
  Artificial sequence
TMHSYGSTNYADSVKG

SEQ ID NO: 56 - protein, 10 aa, Artificial sequence
  Artificial sequence
DDTGWGTVDS

SEQ ID NO: 57 - protein, 118 aa, Artificial sequence
  Artificial sequence
QLQLVESGGGLVQPGGSLRLSCVVSGSIFAINTMGWYRQAPGKQRELVATMHSYGSTNYADSVKGRFTISRDNAKKTVYLQMNSLKPADTAVYYCHADDTGWGTVDSWGQGTQVTVSS

SEQ ID NO: 58 - protein, 10 aa, Artificial sequence
  Artificial sequence
GSIFSINTMG

SEQ ID NO: 59 - protein, 16 aa, Artificial sequence
  Artificial sequence
TMTSHGSTNYADSVKG

SEQ ID NO: 60 - protein, 10 aa, Artificial sequence
  Artificial sequence
NDMGWGTVDA

SEQ ID NO: 61 - protein, 118 aa, Artificial sequence
  Artificial sequence
QLQLVESGGGLVQPGGSLRLSCAASGSIFSINTMGWYRQAPGKQRELVATMTSHGSTNYADSVKGRFTISRDNSKNTVYLQMNSLKLQDTAVYYCNANDMGWGTVDAWGQGTLVTVSS

SEQ ID NO: 62 - protein, 10 aa, Artificial sequence
  Artificial sequence
GSIFSINTMG

SEQ ID NO: 63 - protein, 16 aa, Artificial sequence
  Artificial sequence
TMHSTGSTNYADSVKG

SEQ ID NO: 64 - protein, 10 aa, Artificial sequence
  Artificial sequence
DDMGWGTVDS

SEQ ID NO: 65 - protein, 118 aa, Artificial sequence
  Artificial sequence
QLQLVESGGGLVQPGGSLRLSCAASGSIFSINTMGWYRQAPGKQRELVATMHSTGSTNYADSVKGRFTISRDNAKKTVYLQMNSLKPDDTAVYYCHVDDMGWGTVDSWGQGTQVTVSS

SEQ ID NO: 66 - protein, 10 aa, Artificial sequence
  Artificial sequence
GSIFSINGMG

SEQ ID NO: 67 - protein, 16 aa, Artificial sequence
  Artificial sequence
AITSGGKTDYLDSVKG

SEQ ID NO: 68 - protein, 11 aa, Artificial sequence
  Artificial sequence
YGDVQRGEVRW

SEQ ID NO: 69 - protein, 118 aa, Artificial sequence
  Artificial sequence
QVQLVESGGGLVQPGGSLRLSCAASGSIFSINGMGWYRQAPGKQRELVAAITSGGKTDYLDSVKGRFTISRDSAKNTVALQMNSLKPEDTAVYYCNAYGDVQRGEVRWGQGTQVTVSS

SEQ ID NO: 70 - protein, 10 aa, Artificial sequence
  Artificial sequence
GIIFSINTMG

SEQ ID NO: 71 - protein, 16 aa, Artificial sequence
  Artificial sequence
DISSFGSTNYADSVKG

SEQ ID NO: 72 - protein, 10 aa, Artificial sequence
  Artificial sequence
HDKGWGTVDS

SEQ ID NO: 73 - protein, 118 aa, Artificial sequence
  Artificial sequence
QLQLVESGGGLVQPGGSLRLSCTASGIIFSINTMGWYRQAPGKQRELVADISSFGSTNYADSVKGRFTISRDNAKNSVYLQMNSLKPEDTAVYYCNAHDKGWGTVDSWGQGTQVTVSS

SEQ ID NO: 74 - protein, 10 aa, Artificial sequence
  Artificial sequence
GSIFSINTMG

SEQ ID NO: 75 - protein, 16 aa, Artificial sequence
  Artificial sequence
TMHSTGSTNYADSVKG

SEQ ID NO: 76 - protein, 10 aa, Artificial sequence
  Artificial sequence
DDMGWGTVDS

SEQ ID NO: 77 - protein, 118 aa, Artificial sequence; identical to SEQ ID NO: 65
  Artificial sequence

SEQ ID NO: 78 - protein, 11 aa, Artificial sequence
  Artificial sequence
SIRTFSDYAMA

SEQ ID NO: 79 - protein, 17 aa, Artificial sequence
  Artificial sequence
AISWNGVTTFYADSVKG

SEQ ID NO: 80 - protein, 15 aa, Artificial sequence
  Artificial sequence
GLNVGWGTHEREYDD

SEQ ID NO: 81 - protein, 124 aa, Artificial sequence
  Artificial sequence
QVQLVESGGGLVQAGGSLRLSCAASIRTFSDYAMAWFRQGPRKEREFVAAISWNGVTTFYADSVKGRFTISRDDAKNSVYLQMNSLKPEDTAVYYCAGGLNVGWGTHEREYDDWGQGTQVTVSS

SEQ ID NO: 82 - DNA, 507 bp, Artificial sequence
  Artificial sequence
aagcttgccgccaccatggagacagacacactcctgctatgggtactgctgctctgggttccaggttccaccggtcaggtgcagctcgtggagtctgggggaggcttggtgcagcctggggggtctctgagactctcctgtgcagcctctggattcactttggattattatgccataggctggttccgccaggccccagggaaggagcgtgaggggatctcatgtattaggatttacgatggtaacacatactctgcagagtccgtgaagggccgattcaccatctccagtgacaacgccaagaaccaggtgtatctgcaaatcaacaccctgaaaccggaggacacggccgtttattactgtgcagcagggtcctattactcctgttcagtttaccctgactacgacatggactactggggcaaagggaccctggtcaccgtctcttcaggcagcatggatcctggaggatctcatcatcaccaccaccatcatcactaagaattc

SEQ ID NO: 83 - DNA, 486 bp, Artificial sequence
  Artificial sequence
aagcttgccgccaccatggagacagacacactcctgctatgggtactgctgctctgggttccaggttccaccggtcaggtgcagctcgtggagtctgggggaggcttggtgcagcctggggggtctctgagactctcctgtgcagcctctggacccatcttcagtatcaataccatgggctggtaccgccaggctccagggaagcagcgcgagttggtcgcaactatgcacagtactggtagcacaaactatgcagactccgtgaagggccgattcaccatctccagagacaacgccaagaagacggtgtacctgcaaatgaacagcctgaaacctgacgacacggccgtctattactgtcatgtagatgatacgggttggggaaccgtcgattcctggggccaggggatccaggtcaccgtctcctcgggcagcatggatcctggaggatctcatcatcaccaccaccatcatcactaagaattc

SEQ ID NO: 84 - DNA, 486 bp, Artificial sequence
  Artificial sequence
aagcttgccgccaccatggagacagacacactcctgctatgggtactgctgctctgggttccaggttccaccggtcagttgcagctcgtggagtctgggggaggcttggtgcagcctggggggtctctaagactctcctgtgtagtgtctggaagcatcttcgctatcaataccatgggctggtaccgccaggctccagggaagcagcgcgagttggtcgcaactatgcatagtggtggttccacaaactatgcagactccgtgaaaggccgattcaccatctccagagacgccgccccgaaaacggtgtatctgcaaatgaacagcctgaaacctgcagacacggccgtctattactgtcatgcagacgattcgggttggggaaccgtcgattcgtggggccaggggatccaggtcaccgtctcctcgggcagcatggatcctggaggatctcatcatcaccaccaccatcatcactaagaattc

SEQ ID NO: 85 - DNA, 519 bp, Artificial sequence
  Artificial sequence
aagcttgccgccaccatggagacagacacactcctgctatgggtactgctgctctgggttccaggttccaccggtcaggtgcagctcgtggagtctgggggaggcttggtgcaggctggggggtctctgagactctcctgtgtagcctctggattcacttcggatgattatgtcataggctggttccgccaggccccagggaaggagcgtgagggggtctcatgtattagtagtagtgatggtaccactaactatgcagactccgtgaagggccgattcaccatctccagtgacaacgccaagaacacggtgtatcttcaaatgaacagcctgaaacctgaggacacggccgtttattactgtgcagcagatccaatgcgcgtttgcccttatagtggtacttactatggtatcctggggtttggtacctctggccaggggacccaggtcaccgtctcctcaggcagcatggatcctggaggatctcatcatcaccaccaccatcatcactaagaattc

SEQ ID NO: 86 - DNA, 507 bp, Artificial sequence
  Artificial sequence
aagcttgccgccaccatggagacagacacactcctgctatgggtactgctgctctgggttccaggttccaccggtcagttgcagctcgtggagtctgggggaggcttggtgcaggctggggggtccctgagactctcctgtgcagcctctggactcactttcgaggattacgccataggctggttccgccaggccccagggaaggagcgtgaggggatctcatgtattaggatttacgatggtaacacatactctgcagagtccgtgaagggccgattcaccatctccagtgacaacgccaagaaccaggtgtatctgcaaatcaacaccctgaaaccggaggacacggccgtttattactgtgcagcagggtcctattactcctgttcagtttaccctgactacgacatggactactggggcaaagggaccctggtcaccgtctcctcaggcagcatggatcctggaggatctcatcatcaccaccaccatcatcactaagaattc

SEQ ID NO: 87 - DNA, 507 bp, Artificial sequence
  Artificial sequence
aagcttgccgccaccatggagacagacacactcctgctatgggtactgctgctctgggttccaggttccaccggtcaggtgcagctcgtggagtctgggggaggcttggtgcaggctggggggtccctgagactctcctgtgcagcctctggactcactttcgaggattacgccataggctggttccgccaggccccagggaaggagcgtgaggggatctcatgtattaggatttacgatggtaacacatactctgcagagtccgtgaagggccgattcaccatctccagtgacaacgccaagaaccaggtgtatctgcaaatcaacaccctgaaaccggaggacacggccgtttattactgtgcagcagggtcctattactcctgttcagtttaccctgactacgacatggactactggggcaaagggaccctggtcaccgtctcttcaggcagcatggatcctggaggatctcatcatcaccaccaccatcatcactaagaattc

SEQ ID NO: 88 - DNA, 507 bp, Artificial sequence
  Artificial sequence
aagcttgccgccaccatggagacagacacactcctgctatgggtactgctgctctgggttccaggttccaccggtcaggtgcagctcgtggagtctgggggaggcttggtgcaggctggggggtctctgagactctcctgtgcagcctctggagtcactttcgatgatttagccataggctggttccgccaggtcccagggaaggggcgtgagggggtctcgaccattggtactagtgatggtacggcatactatgcagactccgtgaagggccgattcaccatctccagtgacaacgccaagaatacggtgtatctgcaaatgaacagcctgaaacctgaggacacggccgtttattactgtgcagtggacctagactacgggttggggtccctcctcccgatggggtatgactactggggccaggggacccaggtcaccgtctcctcaggcagcatggatcctggaggatctcatcatcaccaccaccatcatcactaagaattc

SEQ ID NO: 89 - DNA, 519 bp, Artificial sequence
  Artificial sequence
aagcttgccgccaccatggagacagacacactcctgctatgggtactgctgctctgggttccaggttccaccggtcaggtgcagctcgtggagtctgggggaggattggtgcaggctgggggctctctgagagtctcctgtgcagcctctggaggcaccttcagtagtactgccatgggctggttccgccaggctccagggaaggagcgtgagtttgtagcagctattagctggagtggtggctacacatactatgcagactccgtgaggggccgattcaccatctccagagacaacgccctgaacacggtgtctctgcaaatgaacagcctgaaacctgaggacacggccgtttattactgtgcagcagatatctcggggcttgatacggttgcagctggtatctttacggaaccgaacatagactactggggcaaagggaccctggtcaccgtctcctcaggcagcatggatcctggaggatctcatcatcaccaccaccatcatcactaagaattc

SEQ ID NO: 90 - DNA, 486 bp, Artificial sequence
  Artificial sequence
aagcttgccgccaccatggagacagacacactcctgctatgggtactgctgctctgggttccaggttccaccggtcagttgcagctcgtggagtctgggggaggcttggtgcagcctggggggtctctgagactctcctgtgtagtgtctggaagcatcttcgctatcaataccatgggctggtaccgccaggctccagggaagcagcgcgagttggtcgcaactatgcatagttatggtagcacaaactatgcagactccgtgaagggccgattcaccatctccagagacaacgccaagaaaacggtgtatctgcaaatgaacagcctgaaacctgcagacacggccgtctattactgtcatgcagacgatacgggttggggaaccgtcgattcctggggccaggggacccaggtcaccgtctcctcgggcagcatggatcctggaggatctcatcatcaccaccaccatcatcactaagaattc

SEQ ID NO: 91 - DNA, 504 bp, Artificial sequence
  Artificial sequence
aagcttgccgccaccatggagacagacacactcctgctatgggtactgctgctctgggttccaggttccaccggtcaggtgcagctggtggagtctgggggaggattggtgcaggctgggggctctctgagactctcctgtgcggcctctatacgcaccttcagcgactatgccatggcctggttccgccagggtccaaggaaggagcgtgagtttgtggcagcgattagctggaatggtgttacaacattctatgcagactccgtgaagggccgattcaccatctccagagacgacgccaagaactcggtgtatctgcaaatgaacagcctgaaacctgaggacacggccgtttattactgtgcaggaggcctaaatgtgggttggggtacccacgaaagggaatatgacgactggggccaggggacccaggtcaccgtctcctcgggcagcatggatcctggaggatctcatcatcaccaccaccatcatcactaagaattc